European Patent Specification EP 3 257 934 B1, published October 23, 2024. Title: New dibasic organic acid producing strain, preparation and application of same. Applicant: Tianjin Institute of industrial biotechnology, Chinese Academy of Sciences. The sequence listing filed with the application follows.

SEQUENCE LISTING (96 sequences)

SEQ ID NO: 1 - DNA, 1341 bp, Myceliophthora thermophila
atgtacagactcggtcgtagccgcgcattggcgtcggccttcgccgcgcccaaggtttctccctcccccagactccagagcattgcgcaacaacaaaggagagccctgagcatccacgagtaccgctccgccgacctcctccgccagtatggcatcgatattccaaagggcgccgtcgcgacgacggcggctgaggccgaggcggtcgccaagagcatcggcaccgacgacatggtgatcaaggctcaggtgctcgccggcgggcgcggcaagggcagcttcgacaacggcctcaagggcggcgttcgcgtcatctactcgcccaccgaggccaagatgttcgccgagcagatgatcggccacaagctcatcaccaagcagacgggcgccgccggccgtctgtgcaacgccgtctacatctgcgagcgcaagttcgcccgccgcgagttctacctggccgtgctcatggaccgcgcgtcgcagggacccgtcatcgtctcgtcgtcgcagggcggcatggacattgagacggtcgccaaggagaaccccgacgccatcacgaccacctacatcgacatcaacgtgggcgtgacggacgagatcgcgcgcggcatcgccaccaagctgggcttcagcgagcagtgcatcgaggacgccaaggacaccatcaagaacctgtaccgcatcttcctcgagaaggacgcgacccagatcgagatcaacccgctctcggagacgtcggaccacaaggtcatgtgcatggatgccaagttcggctttgacgacaacgccgagttccgccagaaggaggtgttcagctggcgcgacaccacccaggaggacccggaggaggtgcgggccgccgaggccgggctcaacttcatcaagctggacggcgacatcggctgcctggtcaacggcgccggcctggccatggccaccatggacattatcaagctcaacggtgggcagccggccaacttcctcgacgtcggcggcggcgccaccccggcggccatcaaggaggcctttgagctcatcaccagcgaccccaaggtgacggccatctttgtcaacatctttggcggcatcgtgcgctgcgacgccatcgcccacggcctcatcaacacggtcaagtcgctcgacctgaagatccccatcattgcccgcctgcagggcaccaacatggagcaggcccaccagctcatcaacgactcgggcatgaagatcttctccatcgacgacctgcagagcgccgccgagcgcgccgtccagctgtccaaggttgtcaagatggctcgtgacattgacgttggcgtcgagttcaccttgggtatctga

SEQ ID NO: 2 - protein, 446 aa, Myceliophthora thermophila
MYRLGRSRALASAFAAPKVSPSPRLQSIAQQQRRALSIHEYRSADLLRQYGIDIPKGAVATTAAEAEAVAKSIGTDDMVIKAQVLAGGRGKGSFDNGLKGGVRVIYSPTEAKMFAEQMIGHKLITKQTGAAGRLCNAVYICERKFARREFYLAVLMDRASQGPVIVSSSQGGMDIETVAKENPDAITTTYIDINVGVTDEIARGIATKLGFSEQCIEDAKDTIKNLYRIFLEKDATQIEINPLSETSDHKVMCMDAKFGFDDNAEFRQKEVFSWRDTTQEDPEEVRAAEAGLNFIKLDGDIGCLVNGAGLAMATMDIIKLNGGQPANFLDVGGGATPAAIKEAFELITSDPKVTAIFVNIFGGIVRCDAIAHGLINTVKSLDLKIPIIARLQGTNMEQAHQLINDSGMKIFSIDDLQSAAERAVQLSKVVKMARDIDVGVEFTLGI

SEQ ID NO: 3 - DNA, 1564 bp, Myceliophthora thermophila
atggcgccgacgtcaacaacgagcttccccgctgaggtcgtacctcaggcccccgaggaccccctcttcggtctgatgcgggcttacagggctgattccagtccaaacaaggttgatctggtacgccgaaaccccctttcctctctaggggctgtctctgtttgcaagccggctcgcagataagcttaggcaggctaacacgccccgtcccccagggaattggcgcgtatcgtgacgataacgcaaaaccctggattctaccagtggtcaagaaggtgcgcgcattttttcgaggctgacggaatcccaacttcccaattccgaaacgccgtctgccaccggttccggcggcttgggacgcgtcttggacagcagccacgctgcctgcccctcgatcaatttacccgccgccaatccccccaattgcccctcccccgcacaccccctgccgagcagcgagctgacagtttccccggcgtactaggccgatgagattttacgcaacgatccggaagccaaccacgagtaccttccgatcgccggcctcgcatcgctaacaagcaaagccgccgaactcctgctcggtcagtccgcaccggccatcgccgagaagcgcaccgcgtcggttcaaaccatctctggcaccggtgccgtccacctgggcgctctcttcctcgccaaattctacaaagttcagggcgccaaccgcaccgtctacgtcagtaacccgacctgggcgaaccaccaccagatcttcacgaatgtcggcctgcccatcgccacttatccgtacttcaacaagaacaccaaggggctagatatcgatggcatgaaggcggcgcttgagcaggcccctgatgggagcataatcctcctacatgcctgcgcgcacaacccgaccggcgtcgaccctacccctgagcagtggcgcgagattgccctgctgatgaaggccaagagacacttccccttcttcgacacggcttaccagggcttcgcttcgggagacctagaccgggacgccagcgccatcaggctgtttgtcgaggagggcttcgagctggtgattgcccagtcttttgccaaaaacttcggcctctacggcgagcgcgccggttgcttccactacgtggcttccccctctgccgatgccgccagtgtcacgacgcgcgtggcctcgcagctggccattctgcagcgctcggagatcagcaacccccccatctacggcgcccgcatcgcctctatcgttctgaacgacccggcgctgtttgccgagtggcaggagaacctccgcaccatgtcgggccgcattattgacatgcggaagagactccgggccaagctcgaggaactcggcactcctggccagtggaaccatatcacggaccagatcggaatgttcagcttcacggggcttaccgagcctcaggtgctcaagctgcggtccgactaccacatttacatgaccaaaaacgggcgcatcagcatggctggtctgaactcgaaaaatgtcgactacgtcgcaacggctatagataaagtggttcgggaggtgcaatga

SEQ ID NO: 4 - protein, 419 aa, Myceliophthora thermophila
MAPTSTTSFPAEVVPQAPEDPLFGLMRAYRADSSPNKVDLGIGAYRDDNAKPWILPVVKKADEILRNDPEANHEYLPIAGLASLTSKAAELLLGQSAPAIAEKRTASVQTISGTGAVHLGALFLAKFYKVQGANRTVYVSNPTWANHHQIFTNVGLPIATYPYFNKNTKGLDIDGMKAALEQAPDGSIILLHACAHNPTGVDPTPEQWREIALLMKAKRHFPFFDTAYQGFASGDLDRDASAIRLFVEEGFELVIAQSFAKNFGLYGERAGCFHYVASPSADAASVTTRVASQLAILQRSEISNPPIYGARIASIVLNDPALFAEWQENLRTMSGRIIDMRKRLRAKLEELGTPGQWNHITDQIGMFSFTGLTEPQVLKLRSDYHIYMTKNGRISMAGLNSKNVDYVATAIDKVVREVQ

SEQ ID NO: 5 - DNA, 2242 bp, Myceliophthora thermophila
atgtccaaggccgcaactgtcaaggaggccgtgaaggagacgctcgtcggctcgaaagagcccgagaagttttcggcgcagacaagggcgcgcttcaaccgccatgctgtgaaggaccccgagaccggagaattgtatctcggcccggagcaattcatcgacgctattgccccgccgcatgaagactacgtgagtcccttgcgctcagttgctggccaaacctaaggcgcacgtcgcttataccaatccgcatgtagcacaagatcaagcgggaacaatactcgatcctgttccatgttgccgaccgaacaaacaagggcaggctgtcgctcgccgactacgggtacttcgagaacctcctcagcaagcccgatgccgaatatgagatcgcgttccgcctctttgacgtcgagcgcctgggcaccgtgaagtacgaagacttccggcggctttacgaactgaacaagggacccgacagcatcccgttcgactgggactgcgagtgggcaaaactgtacatcggcagcaagtcgaacaggcacagcttgaactaccagcaattctcacagatgctccgcggcttgcagggcgagcgcgttcgacaagctttccagcgcttcgacacggacggcgacgggttcattgagccggaagagtttgcgactatcatccagcagacggccaggcataagctgtcggaccacctgctcgagaacctgcacacgctgtgcaacatttcccagggcagcaaggtgtcgtacgccaatgtccgagcgttcctgaacatgatcaatgagatggatctggtcgagctcatcgtccggcgcgcctgctccaacagcaaggacggccgcatcacgagaaccgagttcctcaaccaggctgctaaaatcacccgcttctccctcttcaccccgatggaggccgatatcctgttccactttgccagcctggatgagccgtcgggaagactgggactcaaggacttcaccaaggtgttggatgcagcgtggcggcggcgcgacgaggaggacgacggccgcgtcgttcctgaggctcggtccactggtcagaatgtcttggcgcagaccatggagtcggcgtacaacttcgctctcggcagtctggctggtgctttcggtgccttcatggtgtacccgatcgatttggtcaagactcggatgcagaaccagcgcggtgccgatccgggccagcgcctgtacaagaactcgatcgactgcttcaagaaggtggtccgcaacgaaggtttcagaggcctgtattcgggtgtcctcccccagcttgtcggtgtcgcgccagagaaagccatcaagcttaccgtgaacgaccttgtccgcgggtggttcaccgataagcagggcaagatccactggggcgccgaggtgctcgctggtggcgccgccggtggttgccaagtggtatgtcattcccgactttgagcccgtacgccatgaggggaaaacaaaagacgctgacgtggactgtgctgcaggtgttcaccaaccccctcgaaattgtcaagattcgcctccaggtgcagggagaggtggccaagagtgtggagggcgcgccgaagcggtcggccatgtggatcgtgcgcaacctcggcctggtcggcctttacaagggcgcgtcggcatgtctgctccgagatgtgccgttttcggccatctacttcccgacctactcccacctgaagcgggacgtctttggggagtcgtcgaccaagaagctcggcgtcctccagctcctcacggctggtgccattgccggcatgcccgcggcatacctgaccacgccgtgcgacgtcatcaagacccgtcttcaagtcgaagcgcgtaagggcgacaccacctatacgggactgcggcacgcggccaagacgatctggaaggaggagggcttccgtgccttcttcaagggcgggcccgctcgtatcttccgttcgtcgccgcagttcggcttcacgctggccgcctatgagctgctgcagagcgtgctcccgttcccgggcaagcagtccgaggccaaggtggcagcgggcgtcgcggaggcgatgtcgaatctcaaggaaaaggccgtcgacagcccgttctaccggtcccgcaacgctctcaagatcctgctcgacttggacgagcactttggccgcacaccgctggggcccaattcacgcggctggaaatcgctgccggggtggatgaacgcaaagacggcgtag

SEQ ID NO: 6 - protein, 699 aa, Myceliophthora thermophila
MSKAATVKEAVKETLVGSKEPEKFSAQTRARFNRHAVKDPETGELYLGPEQFIDAIAPPHEDYHKIKREQYSILFHVADRTNKGRLSLADYGYFENLLSKPDAEYEIAFRLFDVERLGTVKYEDFRRLYELNKGPDSIPFDWDCEWAKLYIGSKSNRHSLNYQQFSQMLRGLQGERVRQAFQRFDTDGDGFIEPEEFATIIQQTARHKLSDHLLENLHTLCNISQGSKVSYANVRAFLNMINEMDLVELIVRRACSNSKDGRITRTEFLNQAAKITRFSLFTPMEADILFHFASLDEPSGRLGLKDFTKVLDAAWRRRDEEDDGRVVPEARSTGQNVLAQTMESAYNFALGSLAGAFGAFMVYPIDLVKTRMQNQRGADPGQRLYKNSIDCFKKVVRNEGFRGLYSGVLPQLVGVAPEKAIKLTVNDLVRGWFTDKQGKIHWGAEVLAGGAAGGCQVVFTNPLEIVKIRLQVQGEVAKSVEGAPKRSAMWIVRNLGLVGLYKGASACLLRDVPFSAIYFPTYSHLKRDVFGESSTKKLGVLQLLTAGAIAGMPAAYLTTPCDVIKTRLQVEARKGDTTYTGLRHAAKTIWKEEGFRAFFKGGPARIFRSSPQFGFTLAAYELLQSVLPFPGKQSEAKVAAGVAEAMSNLKEKAVDSPFYRSRNALKILLDLDEHFGRTPLGPNSRGWKSLPGWMNAKTA

SEQ ID NO: 7 - DNA, 849 bp, Myceliophthora thermophila
atggcgtcagcaaaggagaaggcgccgctgccgttccgctatacgttcatggccggcgccattgccggtgtatctgaaatcctggtcatgtacccgctggatgtcgtgaagacaagagtacagctgcagaccggtaaaggctccggtgccgatgcgtacagtggcatgctcgactgcttccagaagatcatccgcaacgaaggcttctcgaggctctaccgcggcattaccgctcccattctcatggaggcgcccaagcgcgcgaccaagttcgcggccaacgacaaatggggcaaattctacaaggatctctttggccagcagaccatgacacagtcgctctcggtcctgactggtgcttcggccggcgcgactgagtccttcgtcgtggtgcccttcgagctcgtcaagatccgcctccaggacaaggcctcggccggcaagtacagcggtatgattgatgttgtcgtcaagacggtgcgcaacgaaggtctgctggccatgtacaacggcctcgagtctactctctggcgccacattctctggaactcgggctacttcggctgcatcttccaggttcggcaattgctccccaaggcggagacgaagtcgggacaaacaatcaacgacatcgtcgccggtaccattggcggcactgtcggcacgattctgaatacccccatggatgtcgtgaagagccgtatccagaacagcgtcaaggttgccggccaaacacccaagtacaactgggcctggcctgccgtggcgacggttgccaaagaggaaggcttcggggccctctacaaaggcttcatccccaaggttctccggctgggacctggcggcggc

SEQ ID NO: 8 - protein, 304 aa, Myceliophthora thermophila
MASAKEKAPLPFRYTFMAGAIAGVSEILVMYPLDVVKTRVQLQTGKGSGADAYSGMLDCFQKIIRNEGFSRLYRGITAPILMEAPKRATKFAANDKWGKFYKDLFGQQTMTQSLSVLTGASAGATESFVVVPFELVKIRLQDKASAGKYSGMIDVVVKTVRNEGLLAMYNGLESTLWRHILWNSGYFGCIFQVRQLLPKAETKSGQTINDIVAGTIGGTVGTILNTPMDVVKSRIQNSVKVAGQTPKYNWAWPAVATVAKEEGFGALYKGFIPKVLRLGPGGGILLVVYTGVMDFFRKIRDGEA

SEQ ID NO: 9 - DNA, 993 bp, Myceliophthora thermophila
atggtcaaagctgtcgttgctggcgcctccggcggtattggacagccgctgtcgctgctcctgaagctctctccgctcgtcagcgagctcgcactctacgatgttgtcaacacccccggtgttgcgaccgacctgtcgcacatttcatccaacgccaaaaccactggctacctgcccgccaacgacggcgccaagaccgctttcaaggatgccgacatcatcatcatcccggcgggcattccccgcaagcccggcatgacccgtgatgacctcttcaacatcaacgccggcatcgtgaagggcctcattgaggtggccgccgaggtcgcccccaaggccttcatcctggttatttccaaccccgtcaactcgaccgtccccatctcggccgaggtgctcaaggccaagggcgtcttcaacccccagcgcctcttcggtgtcaccaccctcgacattgtccgtgccgagaccttcgttgccgagattgccggcaagagcaacccccaggagttgactgtccccgtcgttggcggtcactccggcgagaccattgttccgcttttcagcaagatcgctccgtctgtcacgattccggacgacaagtacgacgctcttgtcaaccgcgtccagttcggtggtgatgaggttgtcaaggccaaggacggcgctggttctgccacactttcgatggcgtatgctggttacaggttcgccgagaagctcctcaaggccgccgcgggcgtcaagggcctcgttgaaccaagctacgtctaccttcccggcatcccaggtggcaaggagattgccgagaagaccggtgtcgagttcttctccgttcccatcgagcttggccctaatggcgccgagaaggcggtcgatatcctcggcgacatcaccgacaaggagaagaagttgctcgaggcggcagtgtcgggcctgaagcggaacatcaagaagggcatcgacttcgcccacaaccccccccagaagtga

SEQ ID NO: 10 - protein, 330 aa, Myceliophthora thermophila
MVKAVVAGASGGIGQPLSLLLKLSPLVSELALYDVVNTPGVATDLSHISSNAKTTGYLPANDGAKTAFKDADIIIIPAGIPRKPGMTRDDLFNINAGIVKGLIEVAAEVAPKAFILVISNPVNSTVPISAEVLKAKGVFNPQRLFGVTTLDIVRAETFVAEIAGKSNPQELTVPVVGGHSGETIVPLFSKIAPSVTIPDDKYDALVNRVQFGGDEVVKAKDGAGSATLSMAYAGYRFAEKLLKAAAGVKGLVEPSYVYLPGIPGGKEIAEKTGVEFFSVPIELGPNGAEKAVDILGDITDKEKKLLEAAVSGLKRNIKKGIDFAHNPPQK

SEQ ID NO: 11 - DNA, 1143 bp, Aspergillus oryzae
atgctgacacctcccaagtttgaggatgagaagcagctgggccccgtgggtatccgggagaggcttcgccatttcacttgggcctggtacacattaacgatgagtggaggagggctggccgtcctcatcatcagccagccctttgggttccgcggattgagagagatcggcatcgctgtctatatcctcaacctgatcctcttcgcccttgtctgctctaccatggctataaggttcatcctgcacggcaaccttctggagtccctccgtcatgaccgcgagggtctcttcttcccgaccttctggctctccgtcgcaaccatcatctgcggcttgtctcgctacttcggtgaagaatcgaatgagtccttccaactagccctcgaagccctcttctggatctactgcgtctgcaccttactcgtcgcaatcatccaatactcgttcgtcttctcatcccacaagtacggccttcaaaccatgatgccttcatggatccttccagccttccccatcatgctcagcggcaccatcgcctccgtcatcggtgaacaacaacccgctcgcgcagccctccccatcatcggcgccggcgtcaccttccagggcctcggcttctccatcagcttcatgatgtacgcccactacatcggccgactgatggagtccggcctcccccacagcgaccacagaccaggcatgttcatctgcgtcggaccccccgccttcacagccctcgccctcgtcggcatgagcaaaggcctccccgaagacttcaagctgctccacgacgcccacgccctggaagatggccgcatcatcgagctgctggccatctccgccggcgtcttcctctgggccctgagtctctggttcttctgcatcgccattgtcgccgtcatccgctcgccccccgaggccttccacctcaactggtgggccatggtcttccccaacaccggcttcaccctggccaccatcaccctgggcaaggctctcaacagtaacggtgtgaagggcgtcggttccgccatgtctatctgcatcgtgtgcatgtatatcttcgtcttcgtcaacaatgtccgcgccgttatccggaaggatatcatgtacccgggtaaagatgaggatgtatctgattag

SEQ ID NO: 12 - protein, 380 aa, Aspergillus oryzae
MLTPPKFEDEKQLGPVGIRERLRHFTWAWYTLTMSGGGLAVLIISQPFGFRGLREIGIAVYILNLILFALVCSTMAIRFILHGNLLESLRHDREGLFFPTFWLSVATIICGLSRYFGEESNESFQLALEALFWIYCVCTLLVAIIQYSFVFSSHKYGLQTMMPSWILPAFPIMLSGTIASVIGEQQPARAALPIIGAGVTFQGLGFSISFMMYAHYIGRLMESGLPHSDHRPGMFICVGPPAFTALALVGMSKGLPEDFKLLHDAHALEDGRIIELLAISAGVFLWALSLWFFCIAIVAVIRSPPEAFHLNWWAMVFPNTGFTLATITLGKALNSNGVKGVGSAMSICIVCMYIFVFVNNVRAVIRKDIMYPGKDEDVSD

SEQ ID NO: 13 - DNA, 1760 bp, Neurospora crassa
atgggcagccagcctcccatgccgcctcctgtgcagacgggaacgcacgtcatcatccatgacaccacatacaaccagaaccaacagtcgccaacacaacatcaacaacaaaacaggctcaacccagtcgacacctcctttctcggctcccactcccggcagtcctcctccgcaaccgtaaccggtgacgattctgacccatcccgcgccttcggcacctacgccgggacaccaaagggtgagtatgagaagaagggccgctcaaccgattacctctccggccccaccggcgacaactccctcaacacctcggccgcctcctcccggttagccctcaactccaacaacgagaagtccaaccacgatggccacatgtccggcggcgccggccaccaccaccgccgctccgcctccccctcttcctcctcctccgattccgactccgacctggaaggtgccggcggccacatgcagaaaggccatcacaacatagacccctacgatccttcccgcccaaagctaccactcaaagcgcggctaaaacacttcacctgggcctggtacaccctctgcatgtccaccggcggtctctccctcttgatcgccgcgcaaccacacaccttccccggcctgcgccagatcggcatgaccgtatacatcatcaacatcatcatcttcgtcctcctgacctccctccaaatcacccgcttcatgctccacgccggctccttcaaagccagcctcacgcacccgcgcgaaggcttcttcttccccaccttcttcctcagcatcgccactctaatcacctcgacccaaaagtacggcacccctcccgacagcgaacccagccaggacctcgtctgggttttgcacattgccttctggatctacctcatcctcgccaccgccgtcgccatcgggcaatactccttcctcttcagccaaaaacgctccttctccctagccaccatgatgcccacctggatcctgcccatcttccccatcatgctctcgggcaccatcgcggccgtcatctcccccttccagcccccgcaccgcgccatcgtcgtcatctgcgccggcctcacctgccagggcctcggcgccgccgtggcgttcatgatgtacgcacacatggtcggccgtctcatgtccgtcggtcttcccgaccgcgaacaccgtcccggcctgttcatgtgcgttggcccgccgtccttcactgctttggcattcatcggcatggcgcagggcttgccgcgggactttgatcacgacatggacgggttcatcgacgcaggcatgattcgcaccatggctgtcattggcgccgtgtttctctgggcgttagcgttctggtggttctttattggtgtgttggctgtgttggcgagcagacccaagtatttccatttgggatggtgggccagtgttttccccaacacgggattcacgttggcgacgattagtattggaaatgcctttcaaagcgatgcggtgctgtgggtgggcacgggcatgagtttgtgtttgttggggacgtatttgtttgtgttgggcaaccatgtgcgggcggtggtggtgcaggatatttgttatccggggagggatgaggatgtggaggatcattagtgtgggtgggcacgggcatgagtttgtgtttgttggggacgtatttgtttgtgttgggcaaccatgtgcgggcggtggtggtgcaggatatttgttatccggggagggatgaggatgtggaggatcattag

SEQ ID NO: 14 - protein, 542 aa, Neurospora crassa
MGSQPPMPPPVQTGTHVIIHDTTYNQNQQSPTQHQQQNRLNPVDTSFLGSHSRQSSSATVTGDDSDPSRAFGTYAGTPKGEYEKKGRSTDYLSGPTGDNSLNTSAASSRLALNSNNEKSNHDGHMSGGAGHHHRRSASPSSSSSDSDSDLEGAGGHMQKGHHNIDPYDPSRPKLPLKARLKHFTWAWYTLCMSTGGLSLLIAAQPHTFPGLRQIGMTVYIINIIIFVLLTSLQITRFMLHAGSFKASLTHPREGFFFPTFFLSIATLITSTQKYGTPPDSEPSQDLVWVLHIAFWIYLILATAVAIGQYSFLFSQKRSFSLATMMPTWILPIFPIMLSGTIAAVISPFQPPHRAIVVICAGLTCQGLGAAVAFMMYAHMVGRLMSVGLPDREHRPGLFMCVGPPSFTALAFIGMAQGLPRDFDHDMDGFIDAGMIRTMAVIGAVFLWALAFWWFFIGVLAVLASRPKYFHLGWWASVFPNTGFTLATISIGNAFQSDAVLWVGTGMSLCLLGTYLFVLGNHVRAVVVQDICYPGRDEDVEDH

SEQ ID NO: 15 - DNA, 1143 bp, Trichodermareesei
atgaaagcggcattccctcatgccgtcgacataaacgacccgaaccgaccaaagcttcctatccgacagaggcttcagcacttcacatgggcgtggtacactctgcccatgagcacggggggtctctccctgctcatctacgcacagccataccagttcgcgggcgaaagggtgattggcttagtcgtatacattatcaacctcatcatcttttccttggtgacaatggccatgatggctcgcttcttcctacacgccggagagtttgtccggtccatcactcatccccgtgaaggcttcttcgtccccacattcttcctgtctctggccaccatcatcacgagcacgcagcgttatgccataccggacgaccatccgatactggaacctgccgtcaagattgcattctgggtgtacgtcgccctgacggcggttctagccctgggccagtacagctacgtctttgcggcccataacctcagcctcaagaccttcatgccaaccttgattctgcccatcttccccatcatgctttcaggaaccattgcatccgtcatcgcgggcacgcagcccgagttcgatgcgatgcccatcctagtcgccggcctcacctgccagggcctcggcatgtctgtggccatcctcatgtacgcccacatgattgggcgcctgctccagttcggcctgcccaaccgggagcatcgacccggtctcttcatgtgcgtcggtccgccggcatttaccgccttggccctggtcggcatggccaacggcgtgcctgagggcatcagcgagctgggcatcgacaagagcgtcatccaggtcgtggctatcctcgtcgccgtgttcctgtgggcgctgagcttctggtggtttggcattgccgtcattgctgttgtctcgtcgccgccaaagtatttccatctgggctggtgggccatggtgtttcccaacacgggctttacgctggcgacgatttccattgccaaggagttgcttagtcctagtctgcagtgggttactattggtatgagctgctgcatctttaccatcttcatctttgtctttgtgaaccatgttcgtgctgtgatcatccaggacatcatgtatccgggacgagatgagaatgtggaggatcactga

SEQ ID NO: 16 - protein, 380 aa, Trichodermareesei
MKAAFPHAVDINDPNRPKLPIRQRLQHFTWAWYTLPMSTGGLSLLIYAQPYQFAGERVIGLVVYIINLIIFSLVTMAMMARFFLHAGEFVRSITHPREGFFVPTFFLSLATIITSTQRYAIPDDHPILEPAVKIAFWVYVALTAVLALGQYSYVFAAHNLSLKTFMPTLILPIFPIMLSGTIASVIAGTQPEFDAMPILVAGLTCQGLGMSVAILMYAHMIGRLLQFGLPNREHRPGLFMCVGPPAFTALALVGMANGVPEGISELGIDKSVIQVVAILVAVFLWALSFWWFGIAVIAVVSSPPKYFHLGWWAMVFPNTGFTLATISIAKELLSPSLQWVTIGMSCCIFTIFIFVFVNHVRAVIIQDIMYPGRDENVEDH

SEQ ID NO: 17 - DNA, 1251 bp, Myceliophthora thermophila
atgaacgttgaaacgagcctccctggctcgtctggttcggatctggaaaccttccaccatgagaccaagaaacatgccaaccatgattccggaatatctgtcaatcacgaagccgaaataggcgtcaaccatacattcgagaagccaggtccagtggggatccgcgaacgtttacgccattttacctgggcctggtacaccttgaccatgagctgcggcgggttggccctccttattgtcaaccagcctcatgacttcaagggcttgaaggacattgcccgggtagtctactgtctcaaccttgcattcttcgtcatcgtcacttctctcatggccatcagattcatcctgcataagaatatgtgggagtctctcggtcatgaccgtgaaggtctcttcttcccgaccttctggctttccattgcaaccatgatcactggattgtacaagtgcttcggtgatgacgcgaacgagaaatttaccaagtgtctccaagtcctcttctggatctactgtggctgtaccatgatcaccgccgtcggtcagtactcttttgtctttgccacccataaatacgagttgcacaccatgatgccttcgtggattttgcctgccttccctgtcatgcttagtggtaccatcgcgtctgttatcggaagcggccagccagccagtgacggtatccctatcatcatagctggcattaccttccagggacttggtttctcgatcagtttcatgatgtacgcccactacatcggacgactgatggaggtcggcttgccttcccccgaacacaggcctggcatgttcatctgtgttggcccacctgcctttactgccctcgctttggttggtatggctaaggcgttgcctgatgatttccagatcgtcggtgatccccatgctgttattgacggacgcgtcatgctgttcctcgctgtcagtgcggccatcttcctttgggccctgagtttctggtttttctgcattgcggttgttgctgtcgtccgatccccgccgaagggtttccacctcaactggttcgctatggtcttccccaacacgggtttcacccttgccaccatcaccctggccaacatgtttgagagcccaggcgtcaagggcgtggccaccgccatgtctctctgtgtcatcatcatgtttatctttgtcttggttagcgccatccgggccgttatccgcaaggacatcatgtggccgggtcaagatgaggatgtgtctgaatga

SEQ ID NO: 18 - protein, 513 aa, Myceliophthora thermophila
MSTPRRSTYVYSGTGYQPFAVQEDRPLPDPYRSLRGPPPAQAEEAGFQSSQSTIRGSPTASGRSSTEYSESYVGDIEKSLHNDTVPSLPLHSLQSDNGSHDGEQQDKEKYGAPGVEMKSTTTTTGAAADHSGETGARARPKLPIRERLKHFTWAWYTLIMSTGGLSLLMRAQPHQFPGLFQIGLAVFVINIVLFVLVTLAQIARFVLFPGIFARSLGHRREGFFFPTFFLAVATLITCTQRYCVPEDADEARATAGTLLWLLRAAFWTYLLLATCVAVGQYSYVFSAHSFGLQTMMPTWILPIFPVMLSGTIASVIAGSQPPEEAVPIAVAGLTCQGLGIAVAFMMYAHMVGRLMQSGLPDREHRTGLFMCVGPPAFTALAFIGLATGLPQDFDHDMDGFVDAVVIETMGLVGAGFLWALSFWWFGIALLAVLQSPPEHFHLGWWASVFPNTGFVLATISIGKAYHSEGILWLSTALSVVLLLTYLFVLYHHVRAVIVQDIMYPGRDEDVEDH

SEQ ID NO: 19 - DNA, 1143 bp, Aspergillus niger
atgctgacacctcccaagtttgaggatgagaagcagcttggtcccgtgggtatccgggagaggcttcgtcatttcacttgggcctggtacaccttaacaatgagtggaggagggctggccgtcctcatcatcagccagccctttgggttccgcggattgagagagatcggcatcgctgtctacatcctcaacctgatcctcttcgcccttgtctgctctaccatggcgataaggttcatcctgcacggcaaccttctggagtccctccgtcatgaccgcgagggtctcttcttcccgaccttctggctctccgttgcaaccatcatctgcggcctgtctcgctacttcggtgacgaatcgaatgaatccttccaactagccctcgaagccctcttctggatctactgtgtctgcacgttactcgtcgcaatcatccaatactcgttcgtcttctcatcccacaagtacggccttcaaaccatgatgccttcatggatcctcccagccttccccatcatgctcagcggcaccatcgcctccgtcatcggtgaacaacaacccgctcgcgccgccctccccatcatcggcgccggcgtcaccttccagggcctcggcttctccatcagcttcatgatgtacgcccactacatcggccgactgatggagtccggcctcccccacagcgaccacagaccaggcatgttcatctgcatcgggccccctgccttcacagcccctgccctcgtcggcatgagcaaaggcctccccgaagacttcaagctgctccacgacgccaatgctctggaagacggccgtatcatcgagctgctagccatctccgccggcgtcttcctctgggccctgagtctctggttcttctgcatcgccatcgtcgccgtcatccgctcgccccccaaggccttccacctcaactggtgggccatggtcttccccaacaccggcttcaccctggccaccatcaccctgggcaaggctctcaacagtgacggcgtgaagggcgtcggctccgccatgtccatctgcatcgtgtgcatgtacatcttcgtcttcgtcaacaacgtccgcgccgttatccggaaggatatcatgtacccgggtaaagatgaggatgtatctgattag

SEQ ID NO: 20 - protein, 416 aa, Aspergillus niger
MNVETSLPGSSGSDLETFHHETKKHANHDSGISVNHEAEIGVNHTFEKPGPVGIRERLRHFTWAWYTLTMSCGGLALLIVNQPHDFKGLKDIARVVYCLNLAFFVIVTSLMAIRFILHKNMWESLGHDREGLFFPTFWLSIATMITGLYKCFGDDANEKFTKCLQVLFWIYCGCTMITAVGQYSFVFATHKYELHTMMPSWILPAFPVMLSGTIASVIGSGQPASDGIPIIIAGITFQGLGFSISFMMYAHYIGRLMEVGLPSPEHRPGMFICVGPPAFTALALVGMAKALPDDFQIVGDPHAVIDGRVMLFLAVSAAIFLWALSFWFFCIAVVAVVRSPPKGFHLNWFAMVFPNTGFTLATITLANMFESPGVKGVATAMSLCVIIMFIFVLVSAIRAVIRKDIMWPGQDEDVSE

SEQ ID NO: 21 - DNA, 1143 bp, Aspergillus sojae
atgctgacacctcccaagtttgaggatgagaagcagctgggccccgtgggtatccgggagaggcttcgccatttcacttgggcctggtacacattaacgatgagtggaggagggctggccgtcctcatcatcagccagccctttgggttccgcggattgagagagatcggcatcgctgtctatatcctcaacctgatcctcttcgcccttgtctgctctaccatggctataaggttcatcctgcacggcaaccttctggagtccctccgtcatgaccgcgagggtctcttcttcccgaccttctggctctccgtcgcaaccatcatctgcggcttgtctcgctacttcggtgaagaatcgaatgagtccttccaactagccctcgaagccctcttctggatctactgcgtctgcaccttactcgtcgcaatcatccaatactcgttcgtcttctcatcccacaagtacggccttcaaaccatgatgccttcatggatccttccagccttccccatcatgctcagcggcaccatcgcctccgtcatcggtgaacaacaacccgctcgcgcagccctccccatcatcggcgccggcgtcaccttccagggcctcggcttctccatcagcttcatgatgtacgcccactacatcggccgactgatggagtccggcctcccccacagcgaccacagaccaggcatgttcatctgcgtcggaccccccgccttcacagccctcgccctcgtcggcatgagcaaaggcctccccgaagacttcaagctgctccacgacgcccacgccctggaagatggccgcatcatcgagctgctggccatctccgccggcgtcttcctctgggccctgagtctctggttcttctgcatcgccattgtcgccgtcatccgctcgccccccgaggccttccacctcaactggtgggccatggtcttccccaacaccggcttcaccctggccaccatcaccctgggcaaggctctcaacagtaacggcgtgaagggcgtcggctccgccatgtctatctgcatcgtgtgcatgtacatcttcgtctttgtcaacaatgtccgcgccgttatccggaaggatatcatgtacccgggtaaagatgaggatgtatctgattag

SEQ ID NO: 22 - protein, 380 aa, Aspergillus sojae
MLTPPKFEDEKQLGPVGIRERLRHFTWAWYTLTMSGGGLAVLIISQPFGFRGLREIGIAVYILNLILFALVCSTMAIRFILHGNLLESLRHDREGLFFPTFWLSVATIICGLSRYFGDESNESFQLALEALFWIYCVCTLLVAIIQYSFVFSSHKYGLQTMMPSWILPAFPIMLSGTIASVIGEQQPARAALPIIGAGVTFQGLGFSISFMMYAHYIGRLMESGLPHSDHRPGMFICIGPPAFTAPALVGMSKGLPEDFKLLHDANALEDGRIIELLAISAGVFLWALSLWFFCIAIVAVIRSPPKAFHLNWWAMVFPNTGFTLATITLGKALNSDGVKGVGSAMSICIVCMYIFVFVNNVRAVIRKDIMYPGKDEDVSD

SEQ ID NO: 23 - DNA, 30 bp, primer
gctctagacagaagatgatattgaaggagc

SEQ ID NO: 24 - DNA, 32 bp, primer
cccaagcttctattcctttgccctcggacgag

SEQ ID NO: 25 - DNA, 3582 bp, Aspergillus oryzae
atggcggctccgtttcgtcagcctgaggaggcggtcgatgacaccgagttcatcgatgaccaccatgaacacctccgtgataccgtgcaccatcggttgcgcgccaattcctccattatgcacttccagaagatcctcgtcgccaaccgtggtgagatccccattcgtatcttcagaacggcccacgagctgtccttgcagacggttgctatctactctcatgaggatcgactgtcaatgcaccgtcaaaaggccgatgaggcctacatgattggccaccgcggtcagtacacccctgtcggtgcgtacctggcgggcgatgagatcatcaagatcgccctggagcacggtgtccagctgatccacccgggctacggtttcttgtccgagaacgccgacttcgcccgcaaggttgagaacgccggcattgtctttgtgggacccactcccgataccattgacagcttgggtgacaaggtgtcggcccgtcggctggccattaagtgcgaggtccctgtcgttccgggtacggagggccccgtcgagcgctatgaggaggtcaaggcgttcacagacacctatggcttccccatcatcatcaaggctgcctttggcggtggtggccgtggtatgcgtgtggtccgtgaccaggccgagctgcgtgactcgttcgagcgagccacctctgaggcccgctccgccttcggcaatggtaccgtcttcgtcgagcgcttcctcgacaaacccaagcacattgaagtccagcttctgggtgacagccacggcaacgttgtccatctgtttgagcgtgactgctccgtgcagcgtcgtcaccagaaggtcgttgaggttgctccggctaaggacctgccagccgatgtccgggaccgcatcctggccgatgctgtgaagctggccaagtccgtcaactaccgtaacgccggtacagctgagttcctggtggaccagcagaaccgccactacttcattgaaatcaatcctcgtatccaagtcgagcacaccatcaccgaagagattactggtatcgatatcgtggctgcacagatccagattgctgctggtgcaagcctcgagcaactgggcctgactcaggaccgcatctccgcccgcggatttgccattcaatgtcgtatcaccacggaagatcccgccaaggggttctctccggatactggtaagattgaggtttatcgttccgctggtggtaacggtgtccgtctggatggtggtaacggtttcgctggtgctatcatcacccctcactacgactccatgctggtcaagtgtacctgccgtggttcgacctatgaaatcgctcgtcgcaaggttgtgcgtgccttggtcgagttccgtattcgtggtgtgaagaccaacattcccttcctgacttcgcttctgagccacccgaccttcgtcgatggaaactgctggaccactttcatcgacgacacccctgaattgttctctcttgtcggcagtcagaaccgtgcccagaagctgctcgcatacctcggcgatgtagctgtcaacggtagtagcatcaagggccaaattggcgagcccaagctcaagggtgatgtcatcaagccgaagcttttcgatgccgagggcaagccgcttgacgtttccgccccctgcaccaagggttggaagcagattctggaccgggagggtccggctgcctttgcgaaggccgtgcgtgccaacaagggttgcttgatcatggatactacctggcgtgacgcccaccagtctttgctggccacccgtgtgcgtaccatcgacttgttgaacatcgcccatgagaccagctacgcctactccaatgcgtacagtttggaatgctggggtggtgctaccttcgatgtggccatgcgtttcctctatgaggacccctgggaccgcctgcgcaagatgcgtaaggctgttcctaacatcccattccagatgttgctccgtggtgccaacggtgtcgcctactcttccctcccagacaacgccatctaccacttctgtaagcaggctaagaagtgcggtgtcgacattttccgtgttttcgacgccctcaacgatgtcgatcagctcgaggtcggtatcaaggctgttcatgctgccgagggtgttgtcgaggccaccatgtgctacagcggtgacatgctgaacccccacaagaagtacaacctggagtactacatggccttggtggataagattgtagccatgaagcctcacatccttggtatcaaggatatggccggtgtgctgaagccccaggccgctcgcctgttggtgggctccatccgtcagcgctaccctgaccttcccatccacgtccacacccacgactccgctggtactggtgtagcttccatgattgcctgtgcccaggcgggtgccgacgccgtggacgccgcgaccgacagcatgtccggtatgacctcccagcctagcattggtgccattctggcctctcttgagggcactgagcaagaccccggtctcaacctcgcccacgtgcgcgctattgatagctactgggcacagctgcgcttgctctactctcctttcgaggcgggtctcactggccccgaccctgaggtctacgagcacgagatccctggtggtcagttgaccaaccttatcttccaggccagtcagctcggcttgggccagcagtgggccgaaaccaagaaggcctatgaggcggctaatgatttactcggcgacattgtaaaggtcactcccacctccaaggtggtcggtgacttggctcagttcatggtctcgaacaaactgactccagaggatgttgttgagcgtgctggtgagctggacttccctggttctgtgctcgaattcctcgaaggtctcatgggacagcccttcggtggattccccgagccattgcgctcccgcgccctgcgcgatcgccgcaagctcgagaagcgtccaggtctctacctcgagcctttggatttggctaagatcaagagccagatccgtgagaagttcggtgctgctactgagtatgacgtggccagctatgccatgtatcccaaggtcttcgaggactacaagaagttcgtccagaagttcggtgatctctccgtcttgcccacacggtacttcttggccaagcctgagattggcgaggagttccacgttgagctggagaagggtaaggtgctcatcctgaagttgttggccatcggccctctttcagagcagactggtcagcgtgaggtcttctacgaagtcaacggtgaggtgcgccaggtcgctgttgatgacaacaaggcttccgtggacaacacttcacgccctaaggccgatgtgggtgacagcagccaggtcggtgctcctatgagcggtgtggttgttgaaatccgtgtccacgatggtctggaggttaagaagggtgacccacttgccgtcctgagtgccatgaagatggaaatggttatctctgctcctcacagtggaaaggtctccagcttgctggtcaaggagggcgattctgtggatggccaggatctcgtctgcaagatcgtcaaagcgtaa

SEQ ID NO: 26 - protein, 1193 aa, Aspergillus oryzae
MAAPFRQPEEAVDDTEFIDDHHEHLRDTVHHRLRANSSIMHFQKILVANRGEIPIRIFRTAHELSLQTVAIYSHEDRLSMHRQKADEAYMIGHRGQYTPVGAYLAGDEIIKIALEHGVQLIHPGYGFLSENADFARKVENAGIVFVGPTPDTIDSLGDKVSARRLAIKCEVPVVPGTEGPVERYEEVKAFTDTYGFPIIIKAAFGGGGRGMRVVRDQAELRDSFERATSEARSAFGNGTVFVERFLDKPKHIEVQLLGDSHGNVVHLFERDCSVQRRHQKVVEVAPAKDLPADVRDRILADAVKLAKSVNYRNAGTAEFLVDQQNRHYFIEINPRIQVEHTITEEITGIDIVAAQIQIAAGASLEQLGLTQDRISARGFAIQCRITTEDPAKGFSPDTGKIEVYRSAGGNGVRLDGGNGFAGAIITPHYDSMLVKCTCRGSTYEIARRKVVRALVEFRIRGVKTNIPFLTSLLSHPTFVDGNCWTTFIDDTPELFSLVGSQNRAQKLLAYLGDVAVNGSSIKGQIGEPKLKGDVIKPKLFDAEGKPLDVSAPCTKGWKQILDREGPAAFAKAVRANKGCLIMDTTWRDAHQSLLATRVRTIDLLNIAHETSYAYSNAYSLECWGGATFDVAMRFLYEDPWDRLRKMRKAVPNIPFQMLLRGANGVAYSSLPDNAIYHFCKQAKKCGVDIFRVFDALNDVDQLEVGIKAVHAAEGVVEATMCYSGDMLNPHKKYNLEYYMALVDKIVAMKPHILGIKDMAGVLKPQAARLLVGSIRQRYPDLPIHVHTHDSAGTGVASMIACAQAGADAVDAATDSMSGMTSQPSIGAILASLEGTEQDPGLNLAHVRAIDSYWAQLRLLYSPFEAGLTGPDPEVYEHEIPGGQLTNLIFQASQLGLGQQWAETKKAYEAANDLLGDIVKVTPTSKVVGDLAQFMVSNKLTPEDVVERAGELDFPGSVLEFLEGLMGQPFGGFPEPLRSRALRDRRKLEKRPGLYLEPLDLAKIKSQIREKFGAATEYDVASYAMYPKVFEDYKKFVQKFGDLSVLPTRYFLAKPEIGEEFHVELEKGKVLILKLLAIGPLSEQTGQREVFYEVNGEVRQVAVDDNKASVDNTSRPKADVGDSSQVGAPMSGVVVEIRVHDGLEVKKGDPLAVLSAMKMEMVISAPHSGKVSSLLVKEGDSVDGQDLVCKIVKA

SEQ ID NO: 27 - DNA, 1026 bp, Myceliophthora thermophila
atgaaaaagcctgaactcaccgcgacgtctgtcgagaagtttctgatcgaaaagttcgacagcgtctccgacctgatgcagctctcggagggcgaagaatctcgtgctttcagcttcgatgtaggagggcgtggatatgtcctgcgggtaaatagctgcgccgatggtttctacaaagatcgttatgtttatcggcactttgcatcggccgcgctcccgattccggaagtgcttgacattggggaattcagcgagagcctgacctattgcatctcccgccgtgcacagggtgtcacgttgcaagacctgcctgaaaccgaactgcccgctgttctgcagccggtcgcggaggccatggatgcgatcgctgcggccgatcttagccagacgagcgggttcggcccattcggaccgcaaggaatcggtcaatacactacatggcgtgatttcatatgcgcgattgctgatccccatgtgtatcactggcaaactgtgatggacgacaccgtcagtgcgtccgtcgcgcaggctctcgatgagctgatgctttgggccgaggactgccccgaagtccggcacctcgtgcacgcggatttcggctccaacaatgtcctgacggacaatggccgcataacagcggtcattgactggagcgaggcgatgttcggggattcccaatacgaggtcgccaacatcttcttctggaggccgtggttggcttgtatggagcagcagacgcgctacttcgagcggaggcatccggagcttgcaggatcgccgcggctccgggcgtatatgctccgcattggtcttgaccaactctatcagagcttggttgacggcaatttcgatgatgcagcttgggcgcagggtcgatgcgacgcaatcgtccgatccggagccgggactgtcgggcgtacacaaatcgcccgcagaagcgcggccgtctggaccgatggctgtgtagaagtactcgccgatagtggaaaccgacgccccagcactcgtccgagggcaaaggaatag

SEQ ID NO: 28 - DNA, 989 bp, Myceliophthora thermophila
catgtaccttgacgtcctccgaggttcgacatcagggttcgtcatagggagtgaaacacccgccatgattccgtagccgcgcgcgaagatacgaagcagatatttcacggacatggcggagatacttgtttcccgtactaaggtagtcatgtcggagacatctgaacgacagagctggccaagagaaccgaccagttgccccaggacgatctagacaaaaaaaaagagagatgagtgggccacttttgccacaacatcgacggccctgcgaccgcccccaggcaaacaaacaaaccgccgaacaataatacttttgtcattttaggaggagcgttgtatggataaaaacaacatctcgttgctgcagaatgtggacttcaaacttgcagaaaatgggaggcggatttgcatgatcggagggtagttgactcacgccgcaggctgcaaatccgtcctccattattccatgaacaacttcgtaaggttgggctgagcgccaatgcctaacggaccgggggccacagcgcaacgtcccacttaaaggccagcgtgacatgccagttccataccaagtagtggcaccagaggcggccaatgctcagtaagggcagggagggaggctcaaacgattggcaaaaagaggggcttgccagttcagttccctgtgcgagcgcgagaggggcagtttcaaatctggaggggtgtgttgcgctggtctgaagagaaagagaagactgtacttaataattgttcaaagagtccatcatcgcgttgcggactcctctagctgtatttagagccctatcattacttgtcgggtgcgaatcaaaataccgggatgcagccctctggcgatttgcatgcggttgtggaggaagtgaagcctgaatcgcggggctgggcggcaaagcacgacgtgaaattcctggcgaaattcgagggcttgccccaccgtggttgaagtttttgtgctgcgtaaccccaccaac

SEQ ID NO: 29 - DNA, 33 bp, primer
ccttaattaacatgtaccttgacgtcctccgag

SEQ ID NO: 30 - DNA, 31 bp, primer
ggactagttctgaagaacgaaactggcgact

SEQ ID NO: 31 - DNA, 30 bp, primer
ccatcgatcatcaagaacctgtaccgcatc

SEQ ID NO: 32 - DNA, 32 bp, primer
gggtttaaaccaatgatggggatcttcaggtc

SEQ ID NO: 33 - DNA, 31 bp, primer
cgcggatcccaatgatggggatcttcaggtc

SEQ ID NO: 34 - DNA, 39 bp, primer
cgcggatccgtttaaaccatcaagaacctgtaccgcatc

SEQ ID NO: 35 - DNA, 29 bp, primer
ggactagtatggcgccgacgtcaacaacg

SEQ ID NO: 36 - DNA, 29 bp, primer
cggaattctcattgcacctcccgaaccac

SEQ ID NO: 37 - DNA, 29 bp, primer
ggactagtatgtccaaggccgcaactgtc

SEQ ID NO: 38 - DNA, 30 bp, primer
cggaattcctacgccgtctttgcgttcatc

SEQ ID NO: 39 - DNA, 34 bp, primer
gctctagatgcttgcaggaactctctgtgaaacc

SEQ ID NO: 40 - DNA, 33 bp, primer
gcgttaaccccacagtttggagagacgacatcg

SEQ ID NO: 41 - DNA, 35 bp, primer
ccttaattaatgtatatacggggcgaatacgaagg

SEQ ID NO: 42 - DNA, 32 bp, primer
cggaattcttcctcctgcaaactcagcttgag

SEQ ID NO: 43 - DNA, 65 bp, primer
ggaagatcttaattaactcgagcggccgcgtttaaacactagtatgctgacacctcccaagtttg

SEQ ID NO: 44 - DNA, 28 bp, primer
atcctaatcagatacatcctcatcttta

SEQ ID NO: 45 - DNA, 30 bp, primer
ggactagtatgggcagccagcctcccatgc

SEQ ID NO: 46 - DNA, 30 bp, primer
cggaattcctaatgatcctccacatcctca

SEQ ID NO: 47 - DNA, 31 bp, primer
ggactagtatgaaagcggcattccctcatgc

SEQ ID NO: 48 - DNA, 32 bp, primer
cggaattctcagtgatcctccacattctcatc

SEQ ID NO: 49 - DNA, 29 bp, primer
cggactagtatgtcaacaccgcggcgaag

SEQ ID NO: 50 - DNA, 30 bp, primer
ccggaattcttaatgatcctccacgtcctc

SEQ ID NO: 51 - DNA, 26 bp, primer
ggactagtatgaacgttgaaacgagc

SEQ ID NO: 52 - DNA, 28 bp, primer
cggaattctcattcagacacatcctcat

SEQ ID NO: 53 - DNA, 36 bp, primer
gctctagaatgctgacacctcccaagtttgaggatg

SEQ ID NO: 54 - DNA, 38 bp, primer
ccttaattaactaatcagatacatcctcatctttaccc

SEQ ID NO: 55 - DNA, 31 bp, primer
gaagatctcatgtaccttgacgtcctccgag

SEQ ID NO: 56 - DNA, 31 bp, primer; identical to SEQ ID NO: 30

SEQ ID NO: 57 - DNA, 31 bp, primer
gggtttaaacatggcggctccgtttcgtcag

SEQ ID NO: 58 - DNA, 32 bp, primer
gggtttaaacttacgctttgacgatcttgcag

SEQ ID NO: 59 - DNA, 31 bp, primer
cggactagtatggtcaaagctgtcgttgctg

SEQ ID NO: 60 - DNA, 30 bp, primer
cgcggatcctcacttctggggggggttgtg

SEQ ID NO: 61 - DNA, 33 bp, primer
ccttaattaagtccagatcatggttgaccggtg

SEQ ID NO: 62 - DNA, 53 bp, primer
gaacctccttcagagaggttcgtgtttaaactgatgtctgctcaagcggggta

SEQ ID NO: 63 - DNA, 52 bp, primer
accccgcttgagcagacatcagtttaaacacgaacctctctgaaggaggttc

SEQ ID NO: 64 - DNA, 34 bp, primer
cccaagcttctaatagggataataagctagggtc

SEQ ID NO: 65 - DNA, 34 bp, primer
ctttctagacgacgttaactgatattgaaggagc

SEQ ID NO: 66 - DNA, 50 bp, primer
cgtgcaatccatcttgttcaatcatttggatgcttgggtagaataggtaa

SEQ ID NO: 67 - DNA, 50 bp, primer
ttacctattctacccaagcatccaaatgattgaacaagatggattgcacg

SEQ ID NO: 68 - DNA, 54 bp, primer
aaaaaaagcttggtaccatcgatgcggccgcccgcggtcagaagaactcgtcaa

SEQ ID NO: 69 - DNA, 1464 bp, Myceliophthora thermophila
tgacggtgcttttcacctctcgatgcccgaaatcgggtctaagctgagtttgatcaaatatgtgactccaacatcgcccccttcggcaaaccccgtcgacacgtgtgtcatccttccattgcaagcgatcactcgcagggcgtgacgatgaacgagatttttgcccggaccgattcgcggatatagcggcagccgaccagccctaccacactgatggccgtgtccctagtgtatgctcccagaaccgcaagcatacactgggcaatgcttggtatgcagttgaggcagctttatgtttccatacccttccacttcggctcggggactcggcggggtcgcggaagtttgacggcagccgtcgggccttaggccgagattaccgtggttgtggcccagttttagccgttcccgtccgtttcctaccggaccatgattttcgtgaaccattgcaatcccgaagcgcatttccgacgttaaggagttacctccgctgcccacaattcatgatcgtggccggctcaaggcagcgtggcggggcatccgtgtcaagctcccaggaggaggtgcgcgatttcaaatccgggccaaaacaggccaagactggctggccaaaaaaaggagcgtagacggcccgggacatcggacgtcagctcgcagccacccaaaaccggtccgatctactcgcttactgtggtagttcaggtacttttgagtagtaaaaacgctacggcagggccggggggttccccggtgacggaggtgcctctgcggtggcgaacatcccacgcactatcgagctacggtgacacctcgtgtcctgttggtcttgcaatgctggggcggcaggaaatgcgtcgcgctcctcccggccaagacctaaaacagacagcgccgcaaagtcgctcactagcaccgcgaaacgaagatgccccacctcaacgcaatctgtgatgcaagcaattgggaaggctcaccccacctcagcgaggggctcaaccatttttattatcagctcatgccaccacaacatgactgttttctttccttgctcatcccacatttgacaaaaatcgtcgattaatctctttccatacaggccgtccgcgctctgataaccacataaaagtctcttcagtcaacagctcaaagctccctcatccctccaggtaagcagccaaagagctcccccacggaccccgcactgcctcatcccgcctgtatcggacctgcgcgacccagcagagaatcccaaacctttgctgcttgctgcccggttccggactgagctgcaacccaagcctttaaaaagctattcccttctcccacggtgtcaactctgtcctatccctccgacatccgttgagctcaacaactccccgaaccttttaccccgcgccgagctacccctccatcaaaccaccctgacagctcgctcactcacctccccacatcacagaaatcaaa

SEQ ID NO: 70 - DNA, 44 bp, primer
tgcagatctttaattaactcgagtgacggtgcttttcacctctc

SEQ ID NO: 71 - DNA, 54 bp, primer
agtggatccgaattcgatatcgtttaaacactagttttgatttctgtgatgtgg

SEQ ID NO: 72 - DNA, 1000 bp, Myceliophthora thermophila
gtctgctgagccgcactcgtagccatctcccccccaccttaatagataacagaaactagacacggtcgtttgtaaaacaagagttcaacctcgtcatacgctgctttcctgacatggacgtctgctaggtgttaatttttctgggctcaccgcgcattgcagaaaaccttagctctgaacttacacctaccacgcacctacgtagttaggagtttcggcaacggcagatgggtcgggagaatggcggcttgtcaacactccctctacaccaccaaggacacccaaaattaaattagctgcggaattttcagccgctgcagccgatatcatgcaatcgaatacgacccttgccagccgcatgccgcctgtcgtcctggatcttgttggcggaggctgccgaagaaacgtcatagggggacatggcgccgtgacgagtgggaatggagacgctttaacaagcaacgctcctgacccggtacctggaattgaagtggggtctggcgcagctcaaccgacctggctaagctctttgacagggtaaataaagggcccgctgggcccctgctcacggtccgacgcgcccggttcttgcctattggggcagcaaaccttggggcagcatccgccccgaacttccgcatcgagctatcacggaggcgggcccggctcacaggctcaacagacggagacggcccgcccgatccgtgaaaagcttagcccccgcgacagcggagcttaacttggcgtaattaaggcatgtatgtatgtatgtacagtactgtgtgtgttccgtacctttatttaaagccagtcagtcgtcttggccccccaaaactgatcgacacacctacctggctgctcttccttgcacaaagcgatcggccgcaagtcttgaaataatactagtagtggagttaccgaattcggtaattagtatacatccaccacaatacactaccacaccaggcctgcagccacccatcgctagccatccgcagcc

SEQ ID NO: 73 - DNA, 1445 bp, Myceliophthora thermophila
tttgagcgctgggcctccttcggcaaacaagttctcagctgtccccaacatccatccactcttgcatatttaagacagaccgaactatcagagcagccaagcgtcagtcggtactcagggccgataccctttcaagcgacccacgaagactggatggactctggaacaagacggctctggcacacgcccatttggttcttggtcttcatgcgcgaagccagtggctctattacacgctcgactactacacacgtggagcagagtgccacgtcctcaagcagagagtggtcagctcgtgagccccgttcaaagtccggggtagcactctcgcggtccggctgcatctcgctcggcatgacttcttgtttctgttctgtcggcgccaccactctgcgcgaggcggccccgtggcgccggaacacacgagttctgattccgtctcctccccctgcctggttgagcaaagatcgacggggaaatcggatgcggcgagccaagcccacgataccaaaatagcatcccacacgtaattaccttggatcaggagatggtggtgtggtgaaaggacggtaattaaacccgttttttctttttttctttttttttttttttttttaccgagcgctgtgggcgttgatctcccgcaccagagtcgatcgcctttttcattgtgagcgcgcatctcatcaaagctcgcacgatcttcgaccgttgcaagacttggcattccggtatttgggattcggaaccgatcgtttccaacccccgcaacccctgcgcagagccaagccgttgcgaaccaacaaagccagaattgggacgggacgtcatccgccgatagcccggtttttgggatcgcggcgcacggcagagccattccgcattgccgcactagtttatccagcatattagccggccccccaaacccaccaatggcccctgccgccgcaccctgttttcggaaggcctgacgcaccccagatccccctttgggtggtatccatgtggggagttggggagtcgcgcgctccgattcttctgttcacggggctgccgccgaggagcgccgagcgtgcttcggcggtgggactcgagaacagaatggaaattggaggactggcggagtcgtcacagctcactgcagtgaaggtttgggtttgcccgggctgcggtgcggatggggaagcccgagttggcgccggccttggtatccgtgggaacgttcatccaggttgccttgcagcccagcgccctgctgggggagagggagtaaagaaggacgtgtgtggatggggcggacggcggacggataccatacctagctatatattatgtatctgcgccgtggcctgtgacaggaaccactcaactcctctgagccttcaggactcttctccccccaaattcctcgacaagtccgactcggtcaggttctgtgtagcaac

SEQ ID NO: 74 - DNA, 500 bp, Myceliophthora thermophila
catcaagaacctgtaccgcatcttcctcgagaaggacgcgacccagatcgagatcaacccgctctcggagacgtcggaccacaaggtcatgtgcatggatgccaagttcggctttgacgacaacgccgagttccgccagaaggaggtgttcagctggcgcgacaccacccaggaggacccggaggaggtgcgggccgccgaggccgggctcaacttcatcaagctggacggcgacatcggctgcctggtcaacggcgccggcctggccatggccaccatggacattatcaagctcaacggtgggcagccggccaacttcctcgacgtcggcggcggcgccaccccggcggccatcaaggaggcctttgagctcatcaccagcgaccccaaggtgacggccatctttgtcaacatctttggcggcatcgtgcgctgcgacgccatcgcccacggcctcatcaacacggtcaagtcgctcgacctgaagatccccatcattg

SEQ ID NO: 75 - DNA, 500 bp, Myceliophthora thermophila
caatgatggggatcttcaggtcgagcgacttgaccgtgttgatgaggccgtgggcgatggcgtcgcagcgcacgatgccgccaaagatgttgacaaagatggccgtcaccttggggtcgctggtgatgagctcaaaggcctccttgatggccgccggggtggcgccgccgccgacgtcgaggaagttggccggctgcccaccgttgagcttgataatgtccatggtggccatggccaggccggcgccgttgaccaggcagccgatgtcgccgtccagcttgatgaagttgagcccggcctcggcggcccgcacctcctccgggtcctcctgggtggtgtcgcgccagctgaacacctccttctggcggaactcggcgttgtcgtcaaagccgaacttggcatccatgcacatgaccttgtggtccgacgtctccgagagcgggttgatctcgatctgggtcgcgtccttctcgaggaagatgcggtacaggttcttgatg

SEQ ID NO: 76 - DNA, 20 bp, primer
agctgtttactcattattac

SEQ ID NO: 77 - DNA, 47 bp, primer
gctctagagttaacgcggccgcgactagatctgtgccaacgccacag

SEQ ID NO: 78 - DNA, 50 bp, primer
cggaattcgtttaaacttaattaaccgacggaattgaggatatcagtcac

SEQ ID NO: 79 - DNA, 30 bp, primer
gctctagaatgggcagccagcctcccatgc

SEQ ID NO: 80 - DNA, 32 bp, primer
ccttaattaactaatgatcctccacatcctca

SEQ ID NO: 81 - DNA, 38 bp, primer; identical to SEQ ID NO: 54

SEQ ID NO: 82 - DNA, 29 bp, primer
ttccaactagtatgctgacacctcccaag

SEQ ID NO: 83 - DNA, 28 bp, primer
aatggttaacctaatcagatacatcctc

SEQ ID NO: 84 - DNA, 1033 bp, Aspeergillus nidulans
gtccagatcatggttgaccggtgcctggatcttcctatagaatcatccttattcgttgacctagctgattctggagtgacccagagggtcatgacttgagcctaaaatccgccgcctccaccatttgtagaaaaatgtgacgaactcgtgagctctgtacagtgaccggtgactctttctggcatgcggagagacggacggacgcagagagaagggctgagtaataagccactggccagacagctctggcggctctgaggtgcagtggatgattattaatccgggaccggccgcccctccgccccgaagtggaaaggctggtgtgcccctcgttgaccaagaatctattgcatcatcggagaatatggagcttcatcgaatcaccggcagtaagcgaaggagaatgtgaagccaggggtgtatagccgtcggcgaaatagcatgccattaacctaggtacagaagtccaattgcttccgatctggtaaaagattcacgagatagtaccttctccgaagtaggtagagcgagtacccggcgcgtaagctccctaattggcccatccggcatctgtagggcgtccaaatatcgtgcctctcctgctttgcccggtgtatgaaaccggaaaggccgctcaggagctggccagcggcgcagaccgggaacacaagctggcagtcgacccatccggtgctctgcactcgacctgctgaggtccctcagtccctggtaggcagctttgccccgtctgtccgcccggtgtgtcggcggggttgacaaggtcgttgcgtcagtccaacatttgttgccatattttcctgctctccccaccagctgctcttttcttttctctttcttttcccatcttcagtatattcatcttcccatccaagaacctttatttcccctaagtaagtactttgctacatccatactccatccttcccatcccttattcctttgaacctttcagttcgagctttcccacttcatcgcagcttgactaacagctaccccgcttgagcagacatca

SEQ ID NO: 85 - DNA, 964 bp, Myceliophthora thermophila
acgaacctctctgaaggaggttctgagacacgcgcgattcttctgtatatagttttatttttcactctggagtgcttcgctccaccagtacataaaccttttttttcacgtaacaaaatggcttcttttcagaccatgtgaaccatcttgatgccttgacctcttcagttctcactttaacgtagttcgcgtttgtctgtatgtcccagttgcatgtagttgagataaatacccctggaagtgggtctgggcctttgtgggacggagccctctttctgtggtctggagagcccgctctctaccgcctaccttcttaccacagtacactactcacacattgctgaactgacccatcataccgtactttatcctgttaattcgtggtgctgtcgactattctatttgctcaaatggagagcacattcatcggcgcagggatacacggtttatggaccccaagagtgtaaggactattattagtaatattatatgcctctaggcgccttaacttcaacaggcgagcactactaatcaacttttggtagacccaattacaaacgaccatacgtgccggaaattttgggattccgtccgctctccccaaccaagctagaagaggcaacgaacagccaatcccggtgctaattaaattatatggttccatttttttaaaaaaatttttttcttcccattttcctctcgcttttctttttcgcatcgtagttgatcaaagtccaagtcaagcgagctatttgtgctatagctcggtggctataatcagtacagcttagagaggctgtaaaggtatgataccacagcagtattcgcgctataagcggcactcctagactaattgttacggtctacagaagtaggtaataaaagcgttaattgttctaaatactagaggcacttagagaagctatctaaatatatattgaccctagcttattatccctattag

SEQ ID NO: 86 - DNA, 368 bp, Aspeergillus nidulans
cgacgttaactgatattgaaggagcattttttgggcttggctggagctagtggaggtcaacaatgaatgcctattttggtttagtcgtccaggcggtgagcacaaaatttgtgtcgtttgacaagatggttcatttaggcaactggtcagatcagccccacttgtagcagtagcggcggcgctcgaagtgtgactcttattagcagacaggaacgaggacattattatcatctgctgcttggtgcacgataacttggtgcgtttgtcaagcaaggtaagtggacgacccggtcataccttcttaagttcgcccttcctccctttatttcagattcaatctgacttacctattctacccaagcatccaa

SEQ ID NO: 87 - DNA, 24 bp, primer
cagactgtgtggttctgcaacagg

SEQ ID NO: 88 - DNA, 23 bp, primer
ggccaacagtacgaagcatttcg

SEQ ID NO: 89 - DNA, 22 bp, primer
atggcgtcagcaaaggagaagg

SEQ ID NO: 90 - DNA, 22 bp, primer
ctacgcctcgccatccctaatc

SEQ ID NO: 91 - DNA, 1372 bp, Myceliophthora thermophila
atggcgtcagcaaaggagaaggcgccgctgccgttccgctatacgttcatggccggtgagcggtttcccaagagcatcccgaagcagccgccgagactcggtcagctaaccaagtacttcaattcaggcgccattgccggtgtatctgaagcacgttgaccaatggctccaacgggcgtcaattctcacgctaacacctagggcgcgcatagatcctggtcatgtaagccctgccatgctcggacgaggtcgcgcgcctcgcctcaattgctaatgctgaacgctcaaacaggtacccgctggatgtcgtgaagacaagagtgtgagacggcacctcccgttcatttgatatcgaccctctctcccggctgacgaccgaaaagacagctgcagaccggtaaaggctccggtgccgatgcgtacagtggcatgctcgactgcttccagaagatcatccgcaacgaagggtatgcgtcaggaacactcggatacatggaaggggtggtggtgttgacattttgggtagcttctcgaggctctaccgcggcattaccgctcccattctcatggaggcgcccaagcgcgcgaccaagttcgcggccaacgacaaatggggcaaattctacaaggatctctttggccagcagaccatgacacagtcgctctcggtcctgactggtgcttcggccggcgcgactgagtccttcgtcgtggtgcccttcgagctcgtcaagatccgcctccaggacaaggcctcggccggcaagtacagcggtatgattgatgttgtcgtcaagacggtgcgcaacgaaggtctgctggccatgtacaacggcctcgagtctactctctggcgccacattctctggaactcgggctacttcggctgcatcttccaggttcggcaattgctccccaaggcggagacgaagtcgggacaaacaatcaacgacatcgtcgccggtaccattggcggcactgtcggcacgattctgaatacccgtacgtgaaagccatcctaactctccctgcgcgccttgaatgagcacgagttccaccgggcagccggctctcttttcccgcatccacctcctctagccctgaaacaagagaacgaaaactgacattatttctagccatggatgtcgtgaagagccgtatccagaacagcgtcaaggttgccggccaaacacccaagtacaactgggcctggcctgccgtggcgacggttgccaaagaggaaggcttcggggccctctacaaaggcttcatccccaaggttctccggctgggacctggcggcggcattctcctcgtcgtctacaccggggtaatggacttcttccgcaagattagggatggcgaggcgtag

SEQ ID NO: 92 - protein, 304 aa, Myceliophthora thermophila; identical to SEQ ID NO: 8

SEQ ID NO: 93 - DNA, 31 bp, primer; identical to SEQ ID NO: 59

SEQ ID NO: 94 - DNA, 30 bp, primer; identical to SEQ ID NO: 60

SEQ ID NO: 95 - DNA, 1599 bp, Neurospora crassa
atgggtctcttctcgaaaaagtcggctgcgccgcagacccaatcacaagatgagatcgatctcgctgctgagcagaaggtcactttccgtgccgtcttcctcggtgttgtcgcctccgtaggtggcttcatgtttggctacgtcagtggtcaaatttctggtttcttcgacatggaagacttcggtcgtcggttcggtaactaccaagacgcggatggctgggtcttctcagcataccgccagggtgctattgtcgccctactccctgctggtgcccttcttggttcgctcgttgccggtagaattgcggatacccttggtcgccgtatcgccatctctgcgtccgcccttttctcctgcatcggaacaattatcgagatcgcctccaccacgcactgggcccagtttgcggtcggtcgtcttatcaccggtattggtatcggtgctctctccgtcgtcgtcccgatgtaccagtctgagtccgcgcccgccatcctccgtggtatcctcgtctcgtgctaccagctcttcatcactcttggtatctggaccgctgagatgatcaactacggtactcacgacctcagcaactccgcctcttggcgtattcccaacggtatctccttcctctgggctttggttctcggtggcggaatattgttccttcctgagtctccccgttatgcctaccgtgttggtcgcgaggacgaggctcgcaacaccattgcccgccttgccggtctcgagcccagcgcccgctctgtcaacatgcaaatcgatgagatccgtatgaagcttgaggaggagaaggctggtgccgacaccaagtggtacgagatcttcggacctgctctgttgcgccgcacccttatcggtatcattcttcagtctggccagcagcttactggtgccaacttcttcttctactacggaaccacgattttcaaggctactggtcttagcgactcttacgttacccagatcattcttggttccgtcaacgctggatgcactgttgctggtctctgggttgtcaagaatgttggccgccgtaaggccctcatcggtggtgccctctggatgaccatgtgcttcttggtctactctttcgtcggaagatttgtgctcgaccccgtcaacccggctagcactcctcaggccggcaacgtcctcattgtcttctcctgcttcttcatcgtcgcctttgccaccacttggggtcctctcgtctgggccgtcgttgctgagctctaccctgctcgctaccgtgctcctgccatggccttggccaccgcttccaactggctgtggaacttcctcatgtccctcttcacgcgccccatcaccgactccattggctacttctatggcttggtgttcgccggatgctgccttgccctcgccgctttcgtttggctctttgtgatcgagtccaaggaccgcacccttgaggagatcgagaccatgtacaaccagaaggtcagccctaggcactccacccactggcacgctgaggtcccttcgggaccgcgggatgcggaggagaagcccgaggttcacagtggttctgcgacaacctcaagccatggagaggtttag

SEQ ID NO: 96 - protein, 532 aa, Neurospora crassa
MGLFSKKSAAPQTQSQDEIDLAAEQKVTFRAVFLGVVASVGGFMFGYVSGQISGFFDMEDFGRRFGNYQDADGWVFSAYRQGAIVALLPAGALLGSLVAGRIADTLGRRIAISASALFSCIGTIIEIASTTHWAQFAVGRLITGIGIGALSVVVPMYQSESAPAILRGILVSCYQLFITLGIWTAEMINYGTHDLSNSASWRIPNGISFLWALVLGGGILFLPESPRYAYRVGREDEARNTIARLAGLEPSARSVNMQIDEIRMKLEEEKAGADTKWYEIFGPALLRRTLIGIILQSGQQLTGANFFFYYGTTIFKATGLSDSYVTQIILGSVNAGCTVAGLWVVKNVGRRKALIGGALWMTMCFLVYSFVGRFVLDPVNPASTPQAGNVLIVFSCFFIVAFATTWGPLVWAVVAELYPARYRAPAMALATASNWLWNFLMSLFTRPITDSIGYFYGLVFAGCCLALAAFVWLFVIESKDRTLEEIETMYNQKVSPRHSTHWHAEVPSGPRDAEEKPEVHSGSATTSSHGEV